European Patent Application EP 4 613 769 A1, published September 10, 2025. Title: Fusion Protein and Use thereof. Applicant: Beijing Changping Laboratory. Application EP. The sequence listing filed with the application follows.

SEQUENCE LISTING (32 sequences)

SEQ ID NO: 1 - protein, 133 aa, synthetic construct [sequence omitted]

SEQ ID NO: 2 - protein, 227 aa, synthetic construct
DKTHTCPPCPAPELLGGPSVFLFPPKPKDTLMISRTPEVTCVVVDVSHEDPEVKFNWYVDGVEVHNAKTKPREEQYNSTYRVVSVLTVLHQDWLNGKEYKCKVSNKALPAPIEKTISKAKGQPREPQVYTLPPSRDELTKNQVSLTCLVKGFYPSDIAVEWESNGQPENNYKTTPPVLDSDGSFFLYSKLTVDKSRWQQGNVFSCSVMHEALHNHYTQKSLSLSPGK

SEQ ID NO: 3 - protein, 226 aa, synthetic construct
KTHTCPPCPAPEAAGGPSVFLFPPKPKDTLMISRTPEVTCVVVDVSHEDPEVKFNWYVDGVEVHNAKTKPREEQYNSTYRVVSVLTVLHQDWLNGKEYKCKVSNKALGAPIEKTISKAKGQPREPQVYTLPPSRDELTKNQVSLTCLVKGFYPSDIAVEWESNGQPENNYKTTPPVLDSDGSFFLYSKLTVDKSRWQQGNVFSCSVMHEALHNHYTQKSLSLSPGK

SEQ ID NO: 4 - protein, 227 aa, synthetic construct
DKTHTCPPCPAPEAAGGPSVFLFPPKPKDTLMISRTPEVTCVVVDVSHEDPEVKFNWYVDGVEVHNAKTKPREEQYNSTYRVVSVLTVLHQDWLNGKEYKCKVSNKALGAPIEKTISKAKGQPREPQVYTLPPCRDELTKNQVSLWCLVKGFYPSDIAVEWESNGQPENNYKTTPPVLDSDGSFFLYSALTVDKSRWQQGNVFSCSVMHEALHNHYTQKSLSLSPGK

SEQ ID NO: 5 - protein, 227 aa, synthetic construct
DKTHTCPPCPAPEAAGGPSVFLFPPKPKDTLMISRTPEVTCVVVDVSHEDPEVKFNWYVDGVEVHNAKTKPREEQYNSTYRVVSVLTVLHQDWLNGKEYKCKVSNKALGAPIEKTISKAKGQPREPQVCTLPPSRDELTKNQVSLSCAVKGFYPSDIAVEWESNGQPENNYKTTPPVLDSDGSFKLVSKLTVDKSRWQQGNVFSCSVMHEALHNHYTQKSLSLSPGK

SEQ ID NO: 6 - protein, 5 aa, synthetic construct
GGGGS

SEQ ID NO: 7 - protein, 218 aa, synthetic construct
AIQLTQSPSSLSASVGDRVTITCRASESVEYYGTSLMQWYQQKPGKAPKLLIYAASNVESGVPSRFSGSGSGTDFTLTISSLQPEDFATYFCQQSRKDPSTFGGGTKVEIKRTVAAPSVFIFPPSDEQLKSGTASVVCLLNNFYPREAKVQWKVDNALQSGNSQESVTEQDSKDSTYSLSSTLTLSKADYEKHKVYACEVTHQGLSSPVTKSFNRGEC

SEQ ID NO: 8 - protein, 221 aa, synthetic construct
QVQLVQSGAEVKKPGSSVKVSCKASGYTFTSYNMHWVRQAPGQGLEWMGDIYPGNGDTSYNQKFKGRVTITADKSTSTVYMELSSLRSEDTAVYYCARVGGAFPMDYWGQGTTVTVSSASTKGPSVFPLAPSSKSTSGGTAALGCLVKDYFPEPVTVSWNSGALTSGVHTFPAVLQSSGLYSLSSVVTVPSSSLGTQTYICNVNHKPSNTKVDKKVEPKSC

SEQ ID NO: 9 - protein, 244 aa, synthetic construct
AIQLTQSPSSLSASVGDRVTITCRASESVEYYGTSLMQWYQQKPGKAPKLLIYAASNVESGVPSRFSGSGSGTDFTLTISSLQPEDFATYFCQQSRKDPSTFGGGTKVEIKGGGGSGGGGSGGGGSQVQLVQSGAEVKKPGSSVKVSCKASGYTFTSYNMHWVRQAPGQGLEWMGDIYPGNGDTSYNQKFKGRVTITADKSTSTVYMELSSLRSEDTAVYYCARVGGAFPMDYWGQGTTVTVSS

SEQ ID NO: 10 - protein, 365 aa, synthetic construct
APTSSSTKKTQLQLEHLLLDLQMILNGINNYKNPKLTRMLTFKFYMPKKATELKHLQCLEEELKPLEEVLNLAQSKNFHLRPRDLISNINVIVLELKGSETTFMCEYADETATIVEFLNRWITFCQSIISTLTGGGGSDKTHTCPPCPAPEAAGGPSVFLFPPKPKDTLMISRTPEVTCVVVDVSHEDPEVKFNWYVDGVEVHNAKTKPREEQYNSTYRVVSVLTVLHQDWLNGKEYKCKVSNKALGAPIEKTISKAKGQPREPQVCTLPPSRDELTKNQVSLSCAVKGFYPSDIAVEWESNGQPENNYKTTPPVLDSDGSFKLVSKLTVDKSRWQQGNVFSCSVMHEALHNHYTQKSLSLSPGK

SEQ ID NO: 11 - protein, 448 aa, synthetic construct
QVQLVQSGAEVKKPGSSVKVSCKASGYTFTSYNMHWVRQAPGQGLEWMGDIYPGNGDTSYNQKFKGRVTITADKSTSTVYMELSSLRSEDTAVYYCARVGGAFPMDYWGQGTTVTVSSASTKGPSVFPLAPSSKSTSGGTAALGCLVKDYFPEPVTVSWNSGALTSGVHTFPAVLQSSGLYSLSSVVTVPSSSLGTQTYICNVNHKPSNTKVDKKVEPKSCDKTHTCPPCPAPEAAGGPSVFLFPPKPKDTLMISRTPEVTCVVVDVSHEDPEVKFNWYVDGVEVHNAKTKPREEQYNSTYRVVSVLTVLHQDWLNGKEYKCKVSNKALGAPIEKTISKAKGQPREPQVYTLPPCRDELTKNQVSLWCLVKGFYPSDIAVEWESNGQPENNYKTTPPVLDSDGSFFLYSALTVDKSRWQQGNVFSCSVMHEALHNHYTQKSLSLSPGK

SEQ ID NO: 12 - protein, 471 aa, synthetic construct
AIQLTQSPSSLSASVGDRVTITCRASESVEYYGTSLMQWYQQKPGKAPKLLIYAASNVESGVPSRFSGSGSGTDFTLTISSLQPEDFATYFCQQSRKDPSTFGGGTKVEIKGGGGSGGGGSGGGGSQVQLVQSGAEVKKPGSSVKVSCKASGYTFTSYNMHWVRQAPGQGLEWMGDIYPGNGDTSYNQKFKGRVTITADKSTSTVYMELSSLRSEDTAVYYCARVGGAFPMDYWGQGTTVTVSSDKTHTCPPCPAPEAAGGPSVFLFPPKPKDTLMISRTPEVTCVVVDVSHEDPEVKFNWYVDGVEVHNAKTKPREEQYNSTYRVVSVLTVLHQDWLNGKEYKCKVSNKALGAPIEKTISKAKGQPREPQVYTLPPCRDELTKNQVSLWCLVKGFYPSDIAVEWESNGQPENNYKTTPPVLDSDGSFFLYSALTVDKSRWQQGNVFSCSVMHEALHNHYTQKSLSLSPGK

SEQ ID NO: 13 - protein, 214 aa, synthetic construct
EIVLTQSPGTLSLSPGERATLSCRASQSVSSYLAWYQQKPGQAPRLLIYGISSRATGIPDRFSGSGSGTDFTLTISSLQPEDFATYYCQQANNFPLTFGGGTKLEIKRTVAAPSVFIFPPSDEQLKSGTASVVCLLNNFYPREAKVQWKVDNALQSGNSQESVTEQDSKDSTYSLSSTLTLSKADYEKHKVYACEVTHQGLSSPVTKSFNRGEC

SEQ ID NO: 14 - protein, 222 aa, synthetic construct
QVQLVQSGAEVKKPGSSVKVSCKASGGTFSSYAISWVRQAPGQGLEWMGGIIPIFGTANYAQKFQGRVTITADESTSTAYMELSSLRSEDTAVYYCAASTLRVPNPPYWGQGTLVTVSSASTKGPSVFPLAPSSKSTSGGTAALGCLVKDYFPEPVTVSWNSGALTSGVHTFPAVLQSSGLYSLSSVVTVPSSSLGTQTYICNVNHKPSNTKVDKKVEPKSC

SEQ ID NO: 15 - protein, 241 aa, synthetic construct
EIVLTQSPGTLSLSPGERATLSCRASQSVSSYLAWYQQKPGQAPRLLIYGISSRATGIPDRFSGSGSGTDFTLTISSLQPEDFATYYCQQANNFPLTFGGGTKLEIKGGGGSGGGGSGGGGSQVQLVQSGAEVKKPGSSVKVSCKASGGTFSSYAISWVRQAPGQGLEWMGGIIPIFGTANYAQKFQGRVTITADESTSTAYMELSSLRSEDTAVYYCAASTLRVPNPPYWGQGTLVTVSS

SEQ ID NO: 16 - protein, 449 aa, synthetic construct
QVQLVQSGAEVKKPGSSVKVSCKASGGTFSSYAISWVRQAPGQGLEWMGGIIPIFGTANYAQKFQGRVTITADESTSTAYMELSSLRSEDTAVYYCAASTLRVPNPPYWGQGTLVTVSSASTKGPSVFPLAPSSKSTSGGTAALGCLVKDYFPEPVTVSWNSGALTSGVHTFPAVLQSSGLYSLSSVVTVPSSSLGTQTYICNVNHKPSNTKVDKKVEPKSCDKTHTCPPCPAPEAAGGPSVFLFPPKPKDTLMISRTPEVTCVVVDVSHEDPEVKFNWYVDGVEVHNAKTKPREEQYNSTYRVVSVLTVLHQDWLNGKEYKCKVSNKALGAPIEKTISKAKGQPREPQVYTLPPCRDELTKNQVSLWCLVKGFYPSDIAVEWESNGQPENNYKTTPPVLDSDGSFFLYSALTVDKSRWQQGNVFSCSVMHEALHNHYTQKSLSLSPGK

SEQ ID NO: 17 - protein, 468 aa, synthetic construct
EIVLTQSPGTLSLSPGERATLSCRASQSVSSYLAWYQQKPGQAPRLLIYGISSRATGIPDRFSGSGSGTDFTLTISSLQPEDFATYYCQQANNFPLTFGGGTKLEIKGGGGSGGGGSGGGGSQVQLVQSGAEVKKPGSSVKVSCKASGGTFSSYAISWVRQAPGQGLEWMGGIIPIFGTANYAQKFQGRVTITADESTSTAYMELSSLRSEDTAVYYCAASTLRVPNPPYWGQGTLVTVSSDKTHTCPPCPAPEAAGGPSVFLFPPKPKDTLMISRTPEVTCVVVDVSHEDPEVKFNWYVDGVEVHNAKTKPREEQYNSTYRVVSVLTVLHQDWLNGKEYKCKVSNKALGAPIEKTISKAKGQPREPQVYTLPPCRDELTKNQVSLWCLVKGFYPSDIAVEWESNGQPENNYKTTPPVLDSDGSFFLYSALTVDKSRWQQGNVFSCSVMHEALHNHYTQKSLSLSPGK

SEQ ID NO: 18 - protein, 609 aa, synthetic construct
AIQLTQSPSSLSASVGDRVTITCRASESVEYYGTSLMQWYQQKPGKAPKLLIYAASNVESGVPSRFSGSGSGTDFTLTISSLQPEDFATYFCQQSRKDPSTFGGGTKVEIKGGGGSGGGGSGGGGSQVQLVQSGAEVKKPGSSVKVSCKASGYTFTSYNMHWVRQAPGQGLEWMGDIYPGNGDTSYNQKFKGRVTITADKSTSTVYMELSSLRSEDTAVYYCARVGGAFPMDYWGQGTTVTVSSDKTHTCPPCPAPEAAGGPSVFLFPPKPKDTLMISRTPEVTCVVVDVSHEDPEVKFNWYVDGVEVHNAKTKPREEQYNSTYRVVSVLTVLHQDWLNGKEYKCKVSNKALGAPIEKTISKAKGQPREPQVYTLPPSRDELTKNQVSLTCLVKGFYPSDIAVEWESNGQPENNYKTTPPVLDSDGSFFLYSKLTVDKSRWQQGNVFSCSVMHEALHNHYTQKSLSLSPGKGGGGSAPTSSSTKKTQLQLEHLLLDLQMILNGINNYKNPKLTLMLTAKFYMPKKATELKHLQCLEEELKPLEEVLNLAQSKNFHLRPRDLISNINVIVLELKGSETTFMCEYADETATIVEFLNRWITFCQSIISTLT

SEQ ID NO: 19 - protein, 614 aa, synthetic construct
APTSSSTKKTQLQLEHLLLDLQMILNGINNYKNPKLTLMLTAKFYMPKKATELKHLQCLEEELKPLEEVLNLAQSKNFHLRPRDLISNINVIVLELKGSETTFMCEYADETATIVEFLNRWITFCQSIISTLTGGGGSDKTHTCPPCPAPEAAGGPSVFLFPPKPKDTLMISRTPEVTCVVVDVSHEDPEVKFNWYVDGVEVHNAKTKPREEQYNSTYRVVSVLTVLHQDWLNGKEYKCKVSNKALGAPIEKTISKAKGQPREPQVYTLPPSRDELTKNQVSLTCLVKGFYPSDIAVEWESNGQPENNYKTTPPVLDSDGSFFLYSKLTVDKSRWQQGNVFSCSVMHEALHNHYTQKSLSLSPGKGGGGSAIQLTQSPSSLSASVGDRVTITCRASESVEYYGTSLMQWYQQKPGKAPKLLIYAASNVESGVPSRFSGSGSGTDFTLTISSLQPEDFATYFCQQSRKDPSTFGGGTKVEIKGGGGSGGGGSGGGGSQVQLVQSGAEVKKPGSSVKVSCKASGYTFTSYNMHWVRQAPGQGLEWMGDIYPGNGDTSYNQKFKGRVTITADKSTSTVYMELSSLRSEDTAVYYCARVGGAFPMDYWGQGTTVTVSS

SEQ ID NO: 20 - protein, 614 aa, synthetic construct
AIQLTQSPSSLSASVGDRVTITCRASESVEYYGTSLMQWYQQKPGKAPKLLIYAASNVESGVPSRFSGSGSGTDFTLTISSLQPEDFATYFCQQSRKDPSTFGGGTKVEIKGGGGSGGGGSGGGGSQVQLVQSGAEVKKPGSSVKVSCKASGYTFTSYNMHWVRQAPGQGLEWMGDIYPGNGDTSYNQKFKGRVTITADKSTSTVYMELSSLRSEDTAVYYCARVGGAFPMDYWGQGTTVTVSSGGGGSAPTSSSTKKTQLQLEHLLLDLQMILNGINNYKNPKLTLMLTAKFYMPKKATELKHLQCLEEELKPLEEVLNLAQSKNFHLRPRDLISNINVIVLELKGSETTFMCEYADETATIVEFLNRWITFCQSIISTLTGGGGSDKTHTCPPCPAPEAAGGPSVFLFPPKPKDTLMISRTPEVTCVVVDVSHEDPEVKFNWYVDGVEVHNAKTKPREEQYNSTYRVVSVLTVLHQDWLNGKEYKCKVSNKALGAPIEKTISKAKGQPREPQVYTLPPSRDELTKNQVSLTCLVKGFYPSDIAVEWESNGQPENNYKTTPPVLDSDGSFFLYSKLTVDKSRWQQGNVFSCSVMHEALHNHYTQKSLSLSPGK

SEQ ID NO: 21 - protein, 609 aa, synthetic construct
APTSSSTKKTQLQLEHLLLDLQMILNGINNYKNPKLTLMLTAKFYMPKKATELKHLQCLEEELKPLEEVLNLAQSKNFHLRPRDLISNINVIVLELKGSETTFMCEYADETATIVEFLNRWITFCQSIISTLTGGGGSAIQLTQSPSSLSASVGDRVTITCRASESVEYYGTSLMQWYQQKPGKAPKLLIYAASNVESGVPSRFSGSGSGTDFTLTISSLQPEDFATYFCQQSRKDPSTFGGGTKVEIKGGGGSGGGGSGGGGSQVQLVQSGAEVKKPGSSVKVSCKASGYTFTSYNMHWVRQAPGQGLEWMGDIYPGNGDTSYNQKFKGRVTITADKSTSTVYMELSSLRSEDTAVYYCARVGGAFPMDYWGQGTTVTVSSDKTHTCPPCPAPEAAGGPSVFLFPPKPKDTLMISRTPEVTCVVVDVSHEDPEVKFNWYVDGVEVHNAKTKPREEQYNSTYRVVSVLTVLHQDWLNGKEYKCKVSNKALGAPIEKTISKAKGQPREPQVYTLPPSRDELTKNQVSLTCLVKGFYPSDIAVEWESNGQPENNYKTTPPVLDSDGSFFLYSKLTVDKSRWQQGNVFSCSVMHEALHNHYTQKSLSLSPGK

SEQ ID NO: 22 - protein, 606 aa, synthetic construct
EIVLTQSPGTLSLSPGERATLSCRASQSVSSYLAWYQQKPGQAPRLLIYGISSRATGIPDRFSGSGSGTDFTLTISSLQPEDFATYYCQQANNFPLTFGGGTKLEIKGGGGSGGGGSGGGGSQVQLVQSGAEVKKPGSSVKVSCKASGGTFSSYAISWVRQAPGQGLEWMGGIIPIFGTANYAQKFQGRVTITADESTSTAYMELSSLRSEDTAVYYCAASTLRVPNPPYWGQGTLVTVSSDKTHTCPPCPAPEAAGGPSVFLFPPKPKDTLMISRTPEVTCVVVDVSHEDPEVKFNWYVDGVEVHNAKTKPREEQYNSTYRVVSVLTVLHQDWLNGKEYKCKVSNKALGAPIEKTISKAKGQPREPQVYTLPPSRDELTKNQVSLTCLVKGFYPSDIAVEWESNGQPENNYKTTPPVLDSDGSFFLYSKLTVDKSRWQQGNVFSCSVMHEALHNHYTQKSLSLSPGKGGGGSAPTSSSTKKTQLQLEHLLLDLQMILNGINNYKNPKLTLMLTAKFYMPKKATELKHLQCLEEELKPLEEVLNLAQSKNFHLRPRDLISNINVIVLELKGSETTFMCEYADETATIVEFLNRWITFCQSIISTLT

SEQ ID NO: 23 - protein, 611 aa, synthetic construct
APTSSSTKKTQLQLEHLLLDLQMILNGINNYKNPKLTLMLTAKFYMPKKATELKHLQCLEEELKPLEEVLNLAQSKNFHLRPRDLISNINVIVLELKGSETTFMCEYADETATIVEFLNRWITFCQSIISTLTGGGGSDKTHTCPPCPAPEAAGGPSVFLFPPKPKDTLMISRTPEVTCVVVDVSHEDPEVKFNWYVDGVEVHNAKTKPREEQYNSTYRVVSVLTVLHQDWLNGKEYKCKVSNKALGAPIEKTISKAKGQPREPQVYTLPPSRDELTKNQVSLTCLVKGFYPSDIAVEWESNGQPENNYKTTPPVLDSDGSFFLYSKLTVDKSRWQQGNVFSCSVMHEALHNHYTQKSLSLSPGKGGGGSEIVLTQSPGTLSLSPGERATLSCRASQSVSSYLAWYQQKPGQAPRLLIYGISSRATGIPDRFSGSGSGTDFTLTISSLQPEDFATYYCQQANNFPLTFGGGTKLEIKGGGGSGGGGSGGGGSQVQLVQSGAEVKKPGSSVKVSCKASGGTFSSYAISWVRQAPGQGLEWMGGIIPIFGTANYAQKFQGRVTITADESTSTAYMELSSLRSEDTAVYYCAASTLRVPNPPYWGQGTLVTVSS

SEQ ID NO: 24 - protein, 611 aa, synthetic construct
EIVLTQSPGTLSLSPGERATLSCRASQSVSSYLAWYQQKPGQAPRLLIYGISSRATGIPDRFSGSGSGTDFTLTISSLQPEDFATYYCQQANNFPLTFGGGTKLEIKGGGGSGGGGSGGGGSQVQLVQSGAEVKKPGSSVKVSCKASGGTFSSYAISWVRQAPGQGLEWMGGIIPIFGTANYAQKFQGRVTITADESTSTAYMELSSLRSEDTAVYYCAASTLRVPNPPYWGQGTLVTVSSGGGGSAPTSSSTKKTQLQLEHLLLDLQMILNGINNYKNPKLTLMLTAKFYMPKKATELKHLQCLEEELKPLEEVLNLAQSKNFHLRPRDLISNINVIVLELKGSETTFMCEYADETATIVEFLNRWITFCQSIISTLTGGGGSDKTHTCPPCPAPEAAGGPSVFLFPPKPKDTLMISRTPEVTCVVVDVSHEDPEVKFNWYVDGVEVHNAKTKPREEQYNSTYRVVSVLTVLHQDWLNGKEYKCKVSNKALGAPIEKTISKAKGQPREPQVYTLPPSRDELTKNQVSLTCLVKGFYPSDIAVEWESNGQPENNYKTTPPVLDSDGSFFLYSKLTVDKSRWQQGNVFSCSVMHEALHNHYTQKSLSLSPGK

SEQ ID NO: 25 - protein, 606 aa, synthetic construct
APTSSSTKKTQLQLEHLLLDLQMILNGINNYKNPKLTLMLTAKFYMPKKATELKHLQCLEEELKPLEEVLNLAQSKNFHLRPRDLISNINVIVLELKGSETTFMCEYADETATIVEFLNRWITFCQSIISTLTGGGGSEIVLTQSPGTLSLSPGERATLSCRASQSVSSYLAWYQQKPGQAPRLLIYGISSRATGIPDRFSGSGSGTDFTLTISSLQPEDFATYYCQQANNFPLTFGGGTKLEIKGGGGSGGGGSGGGGSQVQLVQSGAEVKKPGSSVKVSCKASGGTFSSYAISWVRQAPGQGLEWMGGIIPIFGTANYAQKFQGRVTITADESTSTAYMELSSLRSEDTAVYYCAASTLRVPNPPYWGQGTLVTVSSDKTHTCPPCPAPEAAGGPSVFLFPPKPKDTLMISRTPEVTCVVVDVSHEDPEVKFNWYVDGVEVHNAKTKPREEQYNSTYRVVSVLTVLHQDWLNGKEYKCKVSNKALGAPIEKTISKAKGQPREPQVYTLPPSRDELTKNQVSLTCLVKGFYPSDIAVEWESNGQPENNYKTTPPVLDSDGSFFLYSKLTVDKSRWQQGNVFSCSVMHEALHNHYTQKSLSLSPGK

SEQ ID NO: 26 - protein, 214 aa, synthetic construct
DIQMTQSPASLSASLGETVTIQCRASEDIYSGLAWFQQKPGKSPQLLIYGASSLQDGVPSRFSGSGSGTQYSLKISSMQTEDEGVYFCQQGLKYPPTFGSGTKLEIKRTVAAPSVFIFPPSDEQLKSGTASVVCLLNNFYPREAKVQWKVDNALQSGNSQESVTEQDSKDSTYSLSSTLTLSKADYEKHKVYACEVTHQGLSSPVTKSFNRGEC

SEQ ID NO: 27 - protein, 447 aa, synthetic construct
EVQLVESGGGLVQPGRSLKLSCAASGFTFSDFYMAWVRQAPKKGLEWVASISYEGSSTYYGDSVMGRFTISRDNAKSTLYLQMNSLRSEDTATYYCARQREANWEDWGQGVMVTVSSASTKGPSVFPLAPSSKSTSGGTAALGCLVKDYFPEPVTVSWNSGALTSGVHTFPAVLQSSGLYSLSSVVTVPSSSLGTQTYICNVNHKPSNTKVDKKVEPKSCDKTHTCPPCPAPEAAGGPSVFLFPPKPKDTLMISRTPEVTCVVVDVSHEDPEVKFNWYVDGVEVHNAKTKPREEQYNSTYRVVSVLTVLHQDWLNGKEYKCKVSNKALGAPIEKTISKAKGQPREPQVYTLPPCRDELTKNQVSLWCLVKGFYPSDIAVEWESNGQPENNYKTTPPVLDSDGSFFLYSALTVDKSRWQQGNVFSCSVMHEALHNHYTQKSLSLSPGK

SEQ ID NO: 28 - protein, 473 aa, synthetic construct
SYELTQPPSASVNVGETVKITCSGDQLPKYFADWFHQRSDQTILQVIYDDNKRPSGIPERISGSSSGTTATLTIRDVRAEDEGDYYCFSGYVDSDSKLYVFGSGTQLTVLGGGGSGGGGSGGGGSEVRLLESGGGLVKPEGSLKLSCVASGFTFSDYFMSWVRQAPGKGLEWVAHIYTKSYNYATYYSGSVKGRFTISRDDSRSMVYLQMNNLRTEDTATYYCTRDGSGYPSLDFWGQGTQVTVSSDKTHTCPPCPAPEAAGGPSVFLFPPKPKDTLMISRTPEVTCVVVDVSHEDPEVKFNWYVDGVEVHNAKTKPREEQYNSTYRVVSVLTVLHQDWLNGKEYKCKVSNKALGAPIEKTISKAKGQPREPQVYTLPPCRDELTKNQVSLWCLVKGFYPSDIAVEWESNGQPENNYKTTPPVLDSDGSFFLYSALTVDKSRWQQGNVFSCSVMHEALHNHYTQKSLSLSPGK

SEQ ID NO: 29 - protein, 462 aa, synthetic construct
EIVLTQSPATLSLSPGERATLSCRASQSVSSYLAWYQQKPGQAPRLLIYDASNRATGIPARFSGSGSGTDFTLTISSLEPEDFAVYYCQQSSNWPRTFGQGTKVEIKGGGGSGGGGSGGGGSQVQLVESGGGVVQPGRSLRLDCKASGITFSNSGMHWVRQAPGKGLEWVAVIWYDGSKRYYADSVKGRFTISRDNSKNTLFLQMNSLRAEDTAVYYCATNDDYWGQGTLVTVSSDKTHTCPPCPAPEAAGGPSVFLFPPKPKDTLMISRTPEVTCVVVDVSHEDPEVKFNWYVDGVEVHNAKTKPREEQYNSTYRVVSVLTVLHQDWLNGKEYKCKVSNKALGAPIEKTISKAKGQPREPQVYTLPPCRDELTKNQVSLWCLVKGFYPSDIAVEWESNGQPENNYKTTPPVLDSDGSFFLYSALTVDKSRWQQGNVFSCSVMHEALHNHYTQKSLSLSPGK

SEQ ID NO: 30 - protein, 447 aa, synthetic construct
EVQLVESGGGLVQPGRSLKLSCAASGFTFSDFYMAWVRQAPKKGLEWVASISYEGSSTYYGDSVMGRFTISRDNAKSTLYLQMNSLRSEDTATYYCARQREANWEDWGQGVMVTVSSASTKGPSVFPLAPSSKSTSGGTAALGCLVKDYFPEPVTVSWNSGALTSGVHTFPAVLQSSGLYSLSSVVTVPSSSLGTQTYICNVNHKPSNTKVDKKVEPKSCDKTHTCPPCPAPEAAGGPSVFLFPPKPKDTLMISRTPEVTCVVVDVSHEDPEVKFNWYVDGVEVHNAKTKPREEQYNSTYRVVSVLTVLHQDWLNGKEYKCKVSNKALGAPIEKTISKAKGQPREPQVYTLPPSRDELTKNQVSLTCLVKGFYPSDIAVEWESNGQPENNYKTTPPVLDSDGSFFLYSKLTVDKSRWQQGNVFSCSVMHEALHNHYTQKSLSLSPGK

SEQ ID NO: 31 - protein, 365 aa, synthetic construct; identical to SEQ ID NO: 10

SEQ ID NO: 32 - protein, 133 aa, synthetic construct [sequence omitted]